European Patent Application EP 4 715 061 A1, published March 25, 2026. Title: L-氨基酸连接酶的制备方法及其在二肽合成上的应用. Applicant: 凯莱英生命科学技术（天津）有限公司. The sequence listing filed with the application follows.

SEQUENCE LISTING (2 sequences)

SEQ ID NO: 1 - protein, 473 aa, Bacillus sp
MSKKTVLVIADLGGCPPHMFYESVAASYHIVSYIPRPFAITKGHAELIEKYSIAVIKDRDYFETHPSFEHPDSIYWAHDDYLKSEEEVVDDLVRVASFFKADAITTNNELFIAPMAKAAERLGLRGAGVKAAEKARDKSQMRAAFNAAGVKAVKTQPVTTLADFQQAIEHIGTPLILKPTYLASSIGVTLFHDRAGSDDLFLNVQSYLQTIPVPNAVTYEAPFVAETYLEGAYKDWYQEDGYSDYVSVEGLVVEGEYIPFVIHDKTPQIGFTETAHITPSILDNEAQQIIIEAAKKANEGLGLENCATHTEIKLMKNRETGLIESAARFAGWNMIPNIKKVFGVDMAKLLIDVLVDGKKAELPKELLSGHTHYIADCHLYPQHFKESGHIPAEATHITIDHIHIPQDALVGDTVIVSKSVPSKGTFVDLSLFEAFNGIVSLELKGSSSQDVAVSIRNLQKQAAIHLMDELVKG

SEQ ID NO: 2 - DNA, 1419 bp, synthetic construct
  source 1..1419: mol_type = other DNA
atgtcaaaaaagacagttctagtaatagctgatttgggtggctgcccaccgcacatgttttatgaaagcgttgcggcatcctaccatattgtgagctacataccgcgtccgttcgcaatcactaaaggccacgcagagctgattgaaaaatacagcatcgcggtcatcaaggaccgtgactacttcgaaacccacccgtcttttgaacatccggatagcatttactgggcacacgatgactacctgaagagcgaagaagaggtggtggacgacctggtgcgcgtcgcctcttttttcaaagcggacgcaatcaccaccaataacgagctgttcatcgccccgatggcgaaagcggcggaacgtctgggcctgcgtggtgcgggcgtgaaggctgcggaaaaggctcgcgataagtcccaaatgagagctgcgtttaacgccgcaggtgttaaagctgtgaagacccagccggttaccactctggcggatttccagcaagcaatcgagcacatcggtacgccgctgatcctgaagccgacctacttggcttcctctatcggcgtgaccctgtttcatgaccgcgccggttccgacgatttgttcctgaatgttcagagctacctgcaaaccattccggtgccgaacgcggttacgtacgaggcgcctttcgtggctgaaacgtaccttgagggcgcttataaagactggtatcaagaagatggttatagcgattatgttagcgtcgagggtctcgtagttgagggcgaatatattccgttcgtcattcacgataaaaccccgcagatcggctttactgaaaccgcgcatattaccccgagcatcctggataatgaggcgcagcaaattattatcgaagcggcgaaaaaggcgaacgagggtctgggtttggagaactgcgctacccataccgaaatcaagctgatgaaaaaccgtgaaaccggtttgatcgagagcgcagcgcgttttgcaggctggaatatgattcccaacatcaagaaagttttcggtgttgacatggccaagctgctgattgacgtgctggttgacgggaaaaaggcggagcttccaaaagaattactgagcggtcacacccactatattgcggactgtcatctatatccgcaacattttaaagagtctggtcacatccctgcagaggccacccacatcacgattgatcatattcacatcccgcaggacgcgctggtgggtgataccgttatcgtgtcgaagagcgtaccgagcaaaggcacgtttgttgacctgagtcttttcgaggccttcaacggtattgtgagcttagagttgaagggctcatcgtcccaggacgttgctgtttcgatccgtaatctgcagaaacaggcagccatccacctgatggatgaattggtgaagggc